European Patent Specification EP 3 600 415 B1, published September 17, 2025. Title: Methods for Preventing and Treating Heart Disease. Applicant: Novartis AG Beth Israel Deaconess Medical Center, Inc. The sequence listing filed with the application follows.

SEQUENCE LISTING (194 sequences)

SEQ ID NO: 1 - protein, 10 aa, Artificial
  CDR
GYTFTSSYIN

SEQ ID NO: 2 - protein, 10 aa, Artificial
  CDR
GYTFTSSYIN

SEQ ID NO: 3 - protein, 10 aa, Artificial
  CDR
GYTFTSSYIN

SEQ ID NO: 4 - protein, 10 aa, Artificial
  CDR
GYTFTSSYIN

SEQ ID NO: 5 - protein, 10 aa, Artificial
  CDR
GYTFTSSYIN

SEQ ID NO: 6 - protein, 10 aa, Artificial
  CDR
GYTFTSSYIN

SEQ ID NO: 7 - protein, 10 aa, Artificial
  CDR
GYTFTSSYIN

SEQ ID NO: 8 - protein, 10 aa, Artificial
  CDR
GYTFTSSYIN

SEQ ID NO: 9 - protein, 10 aa, Artificial
  CDR
GYTFTSSYIN

SEQ ID NO: 10 - protein, 10 aa, Artificial
  CDR
GYTFTSSYIN

SEQ ID NO: 11 - protein, 10 aa, Artificial
  CDR
GYTFTSSYIN

SEQ ID NO: 12 - protein, 10 aa, Artificial
  CDR
GYTFTSSYIN

SEQ ID NO: 13 - protein, 10 aa, Artificial
  CDR
GYTFTSSYIN

SEQ ID NO: 14 - protein, 10 aa, Artificial
  CDR
GYTFTSSYIN

SEQ ID NO: 15 - protein, 17 aa, Artificial
  CDR
TINPVSGNTSYAQKFQG

SEQ ID NO: 16 - protein, 17 aa, Artificial
  CDR
TINPVSGNTSYAQKFQG

SEQ ID NO: 17 - protein, 17 aa, Artificial
  CDR
TINPVSGNTSYAQKFQG

SEQ ID NO: 18 - protein, 17 aa, Artificial
  CDR
TINPVSGNTSYAQKFQG

SEQ ID NO: 19 - protein, 17 aa, Artificial
  CDR
MINAPIGTTRYAQKFQG

SEQ ID NO: 20 - protein, 17 aa, Artificial
  CDR
QINAASGMTRYAQKFQG

SEQ ID NO: 21 - protein, 17 aa, Artificial
  CDR
MINAPIGTTRYAQKFQG

SEQ ID NO: 22 - protein, 17 aa, Artificial
  CDR
TINPVSGNTRYAQKFQG

SEQ ID NO: 23 - protein, 17 aa, Artificial
  CDR
TINPVSGSTSYAQKFQG

SEQ ID NO: 24 - protein, 17 aa, Artificial
  CDR
QINAASGMTRYAQKFQG

SEQ ID NO: 25 - protein, 17 aa, Artificial
  CDR
NINAAAGITLYAQKFQG

SEQ ID NO: 26 - protein, 17 aa, Artificial
  CDR
TINPPTGGTYYAQKFQG

SEQ ID NO: 27 - protein, 17 aa, Artificial
  CDR
GINPPAGTTSYAQKFQG

SEQ ID NO: 28 - protein, 17 aa, Artificial
  CDR
NINPATGHADYAQKFQG

SEQ ID NO: 29 - protein, 6 aa, Artificial
  CDR
GGWFDY

SEQ ID NO: 30 - protein, 6 aa, Artificial
  CDR
GGWFDY

SEQ ID NO: 31 - protein, 6 aa, Artificial
  CDR
GGWFDY

SEQ ID NO: 32 - protein, 6 aa, Artificial
  CDR
GGWFDY

SEQ ID NO: 33 - protein, 6 aa, Artificial
  CDR
GGWFDY

SEQ ID NO: 34 - protein, 6 aa, Artificial
  CDR
GGWFDY

SEQ ID NO: 35 - protein, 6 aa, Artificial
  CDR
GGWFDY

SEQ ID NO: 36 - protein, 6 aa, Artificial
  CDR
GGWFDY

SEQ ID NO: 37 - protein, 6 aa, Artificial
  CDR
GGWFDY

SEQ ID NO: 38 - protein, 6 aa, Artificial
  CDR
GGWFDY

SEQ ID NO: 39 - protein, 6 aa, Artificial
  CDR
GGWFDY

SEQ ID NO: 40 - protein, 6 aa, Artificial
  CDR
GGWFDY

SEQ ID NO: 41 - protein, 6 aa, Artificial
  CDR
GGWFDY

SEQ ID NO: 42 - protein, 6 aa, Artificial
  CDR
GGWFDY

SEQ ID NO: 43 - protein, 14 aa, Artificial
  CDR
TGTSSDVGSYNYVN

SEQ ID NO: 44 - protein, 14 aa, Artificial
  CDR
TGTSSDVGSYNYVN

SEQ ID NO: 45 - protein, 14 aa, Artificial
  CDR
TGTSSDVGSYNYVN

SEQ ID NO: 46 - protein, 14 aa, Artificial
  CDR
TGTSSDVGSYNYVN

SEQ ID NO: 47 - protein, 14 aa, Artificial
  CDR
TGTSSDVGSYNYVN

SEQ ID NO: 48 - protein, 14 aa, Artificial
  CDR
TGTSSDVGSYNYVN

SEQ ID NO: 49 - protein, 14 aa, Artificial
  CDR
TGTSSDVGSYNYVN

SEQ ID NO: 50 - protein, 14 aa, Artificial
  CDR
TGTSSDVGSYNYVN

SEQ ID NO: 51 - protein, 14 aa, Artificial
  CDR
TGTSSDVGSYNYVN

SEQ ID NO: 52 - protein, 14 aa, Artificial
  CDR
TGTSSDVGSYNYVN

SEQ ID NO: 53 - protein, 14 aa, Artificial
  CDR
TGTSSDVGSYNYVN

SEQ ID NO: 54 - protein, 14 aa, Artificial
  CDR
TGTSSDVGSYNYVN

SEQ ID NO: 55 - protein, 14 aa, Artificial
  CDR
TGTSSDVGSYNYVN

SEQ ID NO: 56 - protein, 14 aa, Artificial
  CDR
TGTSSDVGSYNYVN

SEQ ID NO: 57 - protein, 11 aa, Artificial
  CDR
LMIYGVSKRPS

SEQ ID NO: 58 - protein, 11 aa, Artificial
  CDR
LMIYGVSKRPS

SEQ ID NO: 59 - protein, 11 aa, Artificial
  CDR
LMIYGVSKRPS

SEQ ID NO: 60 - protein, 11 aa, Artificial
  CDR
LMIYGVSKRPS

SEQ ID NO: 61 - protein, 11 aa, Artificial
  CDR
LMIYGVSKRPS

SEQ ID NO: 62 - protein, 11 aa, Artificial
  CDR
LMIYGVSKRPS

SEQ ID NO: 63 - protein, 11 aa, Artificial
  CDR
LMIYGVSKRPS

SEQ ID NO: 64 - protein, 11 aa, Artificial
  CDR
LMIYGVSKRPS

SEQ ID NO: 65 - protein, 11 aa, Artificial
  CDR
LMIYGVSKRPS

SEQ ID NO: 66 - protein, 11 aa, Artificial
  CDR
LMIYGVSKRPS

SEQ ID NO: 67 - protein, 11 aa, Artificial
  CDR
LMIYGVSKRPS

SEQ ID NO: 68 - protein, 11 aa, Artificial
  CDR
LMIYGVSKRPS

SEQ ID NO: 69 - protein, 11 aa, Artificial
  CDR
LMIYGVSKRPS

SEQ ID NO: 70 - protein, 11 aa, Artificial
  CDR
LMIYGVSKRPS

SEQ ID NO: 71 - protein, 9 aa, Artificial
  CDR
QAWTSKMAG

SEQ ID NO: 72 - protein, 9 aa, Artificial
  CDR
SSYTRMGHP

SEQ ID NO: 73 - protein, 10 aa, Artificial
  CDR
ATYGKGVTPP

SEQ ID NO: 74 - protein, 10 aa, Artificial
  CDR
GTFAGGSYYG

SEQ ID NO: 75 - protein, 9 aa, Artificial
  CDR
QAWTSKMAG

SEQ ID NO: 76 - protein, 9 aa, Artificial
  CDR
QAWTSKMAG

SEQ ID NO: 77 - protein, 10 aa, Artificial
  CDR
GTFAGGSYYG

SEQ ID NO: 78 - protein, 10 aa, Artificial
  CDR
GTFAGGSYYG

SEQ ID NO: 79 - protein, 10 aa, Artificial
  CDR
GTFAGGSYYG

SEQ ID NO: 80 - protein, 10 aa, Artificial
  CDR
GTFAGGSYYG

SEQ ID NO: 81 - protein, 10 aa, Artificial
  CDR
GTFAGGSYYG

SEQ ID NO: 82 - protein, 10 aa, Artificial
  CDR
GTFAGGSYYG

SEQ ID NO: 83 - protein, 10 aa, Artificial
  CDR
GTFAGGSYYG

SEQ ID NO: 84 - protein, 10 aa, Artificial
  CDR
GTFAGGSYYG

SEQ ID NO: 85 - protein, 112 aa, Artificial
  VL
DIALTQPASVSGSPGQSITISCTGTSSDVGSYNYVNWYQQHPGKAPKLMIYGVSKRPSGVSNRFSGSKSGNTASLTISGLQAEDEADYYCQAWTSKMAGVFGGGTKLTVLGQ

SEQ ID NO: 86 - protein, 112 aa, Artificial
  VL
DIALTQPASVSGSPGQSITISCTGTSSDVGSYNYVNWYQQHPGKAPKLMIYGVSKRPSGVSNRFSGSKSGNTASLTISGLQAEDEADYYCSSYTRMGHPVFGGGTKLTVLGQ

SEQ ID NO: 87 - protein, 113 aa, Artificial
  VL
DIALTQPASVSGSPGQSITISCTGTSSDVGSYNYVNWYQQHPGKAPKLMIYGVSKRPSGVSNRFSGSKSGNTASLTISGLQAEDEADYYCATYGKGVTPPVFGGGTKLTVLGQ

SEQ ID NO: 88 - protein, 113 aa, Artificial
  VL
DIALTQPASVSGSPGQSITISCTGTSSDVGSYNYVNWYQQHPGKAPKLMIYGVSKRPSGVSNRFSGSKSGNTASLTISGLQAEDEADYYCGTFAGGSYYGVFGGGTKLTVLGQ

SEQ ID NO: 89 - protein, 112 aa, Artificial; identical to SEQ ID NO: 85
  VL

SEQ ID NO: 90 - protein, 112 aa, Artificial; identical to SEQ ID NO: 85
  VL

SEQ ID NO: 91 - protein, 113 aa, Artificial; identical to SEQ ID NO: 88
  VL

SEQ ID NO: 92 - protein, 113 aa, Artificial; identical to SEQ ID NO: 88
  VL

SEQ ID NO: 93 - protein, 113 aa, Artificial; identical to SEQ ID NO: 88
  VL

SEQ ID NO: 94 - protein, 113 aa, Artificial; identical to SEQ ID NO: 88
  VL

SEQ ID NO: 95 - protein, 113 aa, Artificial; identical to SEQ ID NO: 88
  VL

SEQ ID NO: 96 - protein, 113 aa, Artificial; identical to SEQ ID NO: 88
  VL

SEQ ID NO: 97 - protein, 113 aa, Artificial; identical to SEQ ID NO: 88
  VL

SEQ ID NO: 98 - protein, 113 aa, Artificial; identical to SEQ ID NO: 88
  VL

SEQ ID NO: 99 - protein, 115 aa, Artificial
  VH
QVQLVQSGAEVKKPGASVKVSCKASGYTFTSSYINWVRQAPGQGLEWMGTINPVSGNTSYAQKFQGRVTMTRDTSISTAYMELSSLRSEDTAVYYCARGGWFDYWGQGTLVTVSS

SEQ ID NO: 100 - protein, 115 aa, Artificial; identical to SEQ ID NO: 99
  VH

SEQ ID NO: 101 - protein, 115 aa, Artificial; identical to SEQ ID NO: 99
  VH

SEQ ID NO: 102 - protein, 115 aa, Artificial; identical to SEQ ID NO: 99
  VH

SEQ ID NO: 103 - protein, 115 aa, Artificial
  VH
QVQLVQSGAEVKKPGASVKVSCKASGYTFTSSYINWVRQAPGQGLEWMGMINAPIGTTRYAQKFQGRVTMTRDTSISTAYMELSSLRSEDTAVYYCARGGWFDYWGQGTLVTVSS

SEQ ID NO: 104 - protein, 115 aa, Artificial
  VH
QVQLVQSGAEVKKPGASVKVSCKASGYTFTSSYINWVRQAPGQGLEWMGQINAASGMTRYAQKFQGRVTMTRDTSISTAYMELSSLRSEDTAVYYCARGGWFDYWGQGTLVTVSS

SEQ ID NO: 105 - protein, 115 aa, Artificial; identical to SEQ ID NO: 103
  VH

SEQ ID NO: 106 - protein, 115 aa, Artificial
  VH
QVQLVQSGAEVKKPGASVKVSCKASGYTFTSSYINWVRQAPGQGLEWMGTINPVSGNTRYAQKFQGRVTMTRDTSISTAYMELSSLRSEDTAVYYCARGGWFDYWGQGTLVTVSS

SEQ ID NO: 107 - protein, 115 aa, Artificial
  VH
QVQLVQSGAEVKKPGASVKVSCKASGYTFTSSYINWVRQAPGQGLEWMGTINPVSGSTSYAQKFQGRVTMTRDTSISTAYMELSSLRSEDTAVYYCARGGWFDYWGQGTLVTVSS

SEQ ID NO: 108 - protein, 115 aa, Artificial; identical to SEQ ID NO: 104
  VH

SEQ ID NO: 109 - protein, 115 aa, Artificial
  VH
QVQLVQSGAEVKKPGASVKVSCKASGYTFTSSYINWVRQAPGQGLEWMGNINAAAGITLYAQKFQGRVTMTRDTSISTAYMELSSLRSEDTAVYYCARGGWFDYWGQGTLVTVSS

SEQ ID NO: 110 - protein, 115 aa, Artificial
  VH
QVQLVQSGAEVKKPGASVKVSCKASGYTFTSSYINWVRQAPGQGLEWMGTINPPTGGTYYAQKFQGRVTMTRDTSISTAYMELSSLRSEDTAVYYCARGGWFDYWGQGTLVTVSS

SEQ ID NO: 111 - protein, 115 aa, Artificial
  VH
QVQLVQSGAEVKKPGASVKVSCKASGYTFTSSYINWVRQAPGQGLEWMGGINPPAGTTSYAQKFQGRVTMTRDTSISTAYMELSSLRSEDTAVYYCARGGWFDYWGQGTLVTVSS

SEQ ID NO: 112 - protein, 115 aa, Artificial
  VH
QVQLVQSGAEVKKPGASVKVSCKASGYTFTSSYINWVRQAPGQGLEWMGNINPATGHADYAQKFQGRVTMTRDTSISTAYMELSSLRSEDTAVYYCARGGWFDYWGQGTLVTVSS

SEQ ID NO: 113 - DNA, 336 bp, Artificial
  VL
gatatcgcactgacccagccagcttcagtgagcggctcaccaggtcagagcattaccatctcgtgtacgggtactagcagcgatgttggttcttataattatgtgaattggtaccagcagcatcccgggaaggcgccgaaacttatgatttatggtgtttctaagcgtccctcaggcgtgagcaaccgttttagcggatccaaaagcggcaacaccgcgagcctgaccattagcggcctgcaagcggaagacgaagcggattattattgccaggcttggacttctaagatggctggtgtgtttggcggcggcacgaagttaaccgttcttggccag

SEQ ID NO: 114 - DNA, 336 bp, Artificial
  VL
gatatcgcactgacccagccagcttcagtgagcggctcaccaggtcagagcattaccatctcgtgtacgggtactagcagcgatgttggttcttataattatgtgaattggtaccagcagcatcccgggaaggcgccgaaacttatgatttatggtgtttctaagcgtccctcaggcgtgagcaaccgttttagcggatccaaaagcggcaacaccgcgagcctgaccattagcggcctgcaagcggaagacgaagcggattattattgctcttcttatactcgtatgggtcatcctgtgtttggcggcggcacgaagttaaccgttcttggccag

SEQ ID NO: 115 - DNA, 339 bp, Artificial
  VL
gatatcgcactgacccagccagcttcagtgagcggctcaccaggtcagagcattaccatctcgtgtacgggtactagcagcgatgttggttcttataattatgtgaattggtaccagcagcatcccgggaaggcgccgaaacttatgatttatggtgtttctaagcgtccctcaggcgtgagcaaccgttttagcggatccaaaagcggcaacaccgcgagcctgaccattagcggcctgcaagcggaagacgaagcggattattattgcgctacttatggtaagggtgttactcctcctgtgtttggcggcggcacgaagttaaccgttcttggccag

SEQ ID NO: 116 - DNA, 339 bp, Artificial
  VL
gatatcgcactgacccagccagcttcagtgagcggctcaccaggtcagagcattaccatctcgtgtacgggtactagcagcgatgttggttcttataattatgtgaattggtaccagcagcatcccgggaaggcgccgaaacttatgatttatggtgtttctaagcgtccctcaggcgtgagcaaccgttttagcggatccaaaagcggcaacaccgcgagcctgaccattagcggcctgcaagcggaagacgaagcggattattattgcggtacttttgctggtggttcttattatggtgtgtttggcggcggcacgaagttaaccgttcttggccag

SEQ ID NO: 117 - DNA, 336 bp, Artificial; identical to SEQ ID NO: 113
  VL

SEQ ID NO: 118 - DNA, 336 bp, Artificial; identical to SEQ ID NO: 113
  VL

SEQ ID NO: 119 - DNA, 339 bp, Artificial; identical to SEQ ID NO: 116
  VL

SEQ ID NO: 120 - DNA, 339 bp, Artificial; identical to SEQ ID NO: 116
  VL

SEQ ID NO: 121 - DNA, 339 bp, Artificial; identical to SEQ ID NO: 116
  VL

SEQ ID NO: 122 - DNA, 339 bp, Artificial; identical to SEQ ID NO: 116
  VL

SEQ ID NO: 123 - DNA, 339 bp, Artificial; identical to SEQ ID NO: 116
  VL

SEQ ID NO: 124 - DNA, 339 bp, Artificial
  VL
gatatcgcactgacccagccagcttcagtgagcggctcaccaggtcagagcattaccatctcgtgtactggtactagcagcgatgttggttcttataattatgtgaattggtaccagcagcatcccgggaaggcgccgaaacttatgatttatggtgtttctaagcgtccctcaggcgtgagcaaccgttttagcggatccaaaagcggcaacaccgcgagcctgaccattagcggcctgcaagcggaagacgaagcggattattattgcggtacttttgctggtggttcttattatggtgtgtttggcggcggcacgaagttaaccgttcttggccag

SEQ ID NO: 125 - DNA, 339 bp, Artificial; identical to SEQ ID NO: 116
  VL

SEQ ID NO: 126 - DNA, 339 bp, Artificial; identical to SEQ ID NO: 116
  VL

SEQ ID NO: 127 - DNA, 345 bp, Artificial
  VH
caggtgcaattggttcagagcggcgcggaagtgaaaaaaccgggcgcgagcgtgaaagtgagctgcaaagcctccggatatacctttacttcttcttatattaattgggtccgccaagcccctgggcagggtctcgagtggatgggcactatcaatccggtttctggcaatacgtcttacgcgcagaagtttcagggccgggtgaccatgacccgtgataccagcattagcaccgcgtatatggaactgagcagcctgcgtagcgaagatacggccgtgtattattgcgcgcgtggtggttggtttgattattggggccaaggcaccctggtgacggttagctca

SEQ ID NO: 128 - DNA, 345 bp, Artificial; identical to SEQ ID NO: 127
  VH

SEQ ID NO: 129 - DNA, 345 bp, Artificial; identical to SEQ ID NO: 127
  VH

SEQ ID NO: 130 - DNA, 345 bp, Artificial; identical to SEQ ID NO: 127
  VH

SEQ ID NO: 131 - DNA, 345 bp, Artificial
  VH
caggtgcaattggttcagagcggcgcggaagtgaaaaaaccgggcgcgagcgtgaaagtgagctgcaaagcctccggatatacctttacttcttcttatattaattgggtccgccaagcccctgggcagggtctcgagtggatgggcatgattaatgctcctattggtactactcgttatgctcagaagtttcagggtcgggtgaccatgacccgtgataccagcattagcaccgcgtatatggaactgagcagcctgcgtagcgaagatacggccgtgtattattgcgcgcgtggtggttggtttgattattggggccaaggcaccctggtgacggttagctca

SEQ ID NO: 132 - DNA, 345 bp, Artificial
  VH
caggtgcaattggttcagagcggcgcggaagtgaaaaaaccgggcgcgagcgtgaaagtgagctgcaaagcctccggatatacctttacttcttcttatattaattgggtccgccaagcccctgggcagggtctcgagtggatgggccagattaatgctgcttctggtatgactcgttatgctcagaagtttcagggtcgggtgaccatgacccgtgataccagcattagcaccgcgtatatggaactgagcagcctgcgtagcgaagatacggccgtgtattattgcgcgcgtggtggttggtttgattattggggccaaggcaccctggtgacggttagctca

SEQ ID NO: 133 - DNA, 345 bp, Artificial; identical to SEQ ID NO: 131
  VH

SEQ ID NO: 134 - DNA, 345 bp, Artificial
  VH
caggtgcaattggttcagagcggcgcggaagtgaaaaaaccgggcgcgagcgtgaaagtgagctgcaaagcctccggatatacctttacttcttcttatattaattgggtccgccaagcccctgggcagggtctcgagtggatgggcactatcaatccggtttctggcaatacgcgttacgcgcagaagtttcagggccgggtgaccatgacccgtgataccagcattagcaccgcgtatatggaactgagcagcctgcgtagcgaagatacggccgtgtattattgcgcgcgtggtggttggtttgattattggggccaaggcaccctggtgacggttagctca

SEQ ID NO: 135 - DNA, 345 bp, Artificial
  VH
caggtgcaattggttcagagcggcgcggaagtgaaaaaaccgggcgcgagcgtgaaagtgagctgcaaagcctccggatatacctttacttcttcttatattaattgggtccgccaagcccctgggcagggtctcgagtggatgggcactatcaatccggtttctggctctacgtcttacgcgcagaagtttcagggccgggtgaccatgacccgtgataccagcattagcaccgcgtatatggaactgagcagcctgcgtagcgaagatacggccgtgtattattgcgcgcgtggtggttggtttgattattggggccaaggcaccctggtgacggttagctca

SEQ ID NO: 136 - DNA, 345 bp, Artificial
  VH
caggtgcaattggttcagagcggcgcggaagtgaaaaaaccgggcgcgagcgtgaaagtgagctgcaaagcctccggatatacctttacttcttcttatattaattgggtccgccaagcccctgggcagggtctcgagtggatgggccagattaatgctgcttctggtatgactcgttatgctcagaagtttcagggtcgggtcaccatgacccgtgataccagcattagcaccgcgtatatggaactgagcagcctgcgtagcgaagatacggccgtgtattattgcgcgcgtggtggttggtttgattattggggccaaggcaccctggtgacggttagctca

SEQ ID NO: 137 - DNA, 345 bp, Artificial
  VH
caggtgcaattggttcagagcggcgcggaagtgaaaaaaccgggcgcgagcgtgaaagtgagctgcaaagcctccggatatacctttacttcttcttatattaattgggtccgccaagcccctgggcagggtctcgagtggatgggcaatattaatgctgctgctggtattactctttatgctcagaagtttcagggtcgggtcaccatgacccgtgataccagcattagcaccgcgtatatggaactgagcagcctgcgtagcgaagatacggccgtgtattattgcgcgcgtggtggttggtttgattattggggccaaggcaccctggtgacggttagctca

SEQ ID NO: 138 - DNA, 345 bp, Artificial
  VH
caggtgcaattggttcagagcggcgcggaagtgaaaaaaccgggcgcgagcgtgaaagtgagctgcaaagcctccggatatacctttacttcttcttatattaattgggtccgccaagcccctgggcagggtctcgagtggatgggcactattaatcctcctactggaggtacttattatgctcagaagtttcagggtcgggtgaccatgacccgtgataccagcattagcaccgcgtatatggaactgagcagcctgcgtagcgaagatacggccgtgtattattgcgcgcgtggtggttggtttgattattggggccaaggcaccctggtgacggttagctca

SEQ ID NO: 139 - DNA, 345 bp, Artificial
  VH
caggtgcaattggttcagagcggcgcggaagtgaaaaaaccgggcgcgagcgtgaaagtgagctgcaaagcctccggatatacctttacttcttcttatattaattgggtccgccaagcccctgggcagggtctcgagtggatgggcggtattaatcctcctgctggtactacttcttatgctcagaagtttcagggtcgggtcaccatgacccgtgataccagcattagcaccgcgtatatggaactgagcagcctgcgtagcgaagatacggccgtgtattattgcgcgcgtggtggttggtttgattattggggccaaggcaccctggtgacggttagctca

SEQ ID NO: 140 - DNA, 345 bp, Artificial
  VH
caggtgcaattggttcagagcggcgcggaagtgaaaaaaccgggcgcgagcgtgaaagtgagctgcaaagcctccggatatacctttacttcttcttatattaattgggtccgccaagcccctgggcagggtctcgagtggatgggcaatattaatcctgctactggtcatgctgattatgctcagaagtttcagggtcgggtgaccatgacccgtgataccagcattagcaccgcgtatatggaactgagcagcctgcgtagcgaagatacggccgtgtattattgcgcgcgtggtggttggtttgattattggggccaaggcaccctggtgacggttagctca

SEQ ID NO: 141 - protein, 217 aa, Artificial
  light chain
QSALTQPASVSGSPGQSITISCTGTSSDVGSYNYVNWYQQHPGKAPKLMIYGVSKRPSGVSNRFSGSKSGNTASLTISGLQAEDEADYYCGTFAGGSYYGVFGGGTKLTVLGQPKAAPSVTLFPPSSEELQANKATLVCLISDFYPGAVTVAWKADSSPVKAGVETTTPSKQSNNKYAASSYLSLTPEQWKSHRSYSCQVTHEGSTVEKTVAPTECS

SEQ ID NO: 142 - protein, 217 aa, Artificial; identical to SEQ ID NO: 141
  light chain

SEQ ID NO: 143 - protein, 217 aa, Artificial; identical to SEQ ID NO: 141
  light chain

SEQ ID NO: 144 - protein, 217 aa, Artificial; identical to SEQ ID NO: 141
  light chain

SEQ ID NO: 145 - protein, 217 aa, Artificial; identical to SEQ ID NO: 141
  light chain

SEQ ID NO: 146 - protein, 445 aa, Artificial
  heavy chain
QVQLVQSGAEVKKPGASVKVSCKASGYTFTSSYINWVRQAPGQGLEWMGTINPVSGSTSYAQKFQGRVTMTRDTSISTAYMELSRLRSDDTAVYYCARGGWFDYWGQGTLVTVSSASTKGPSVFPLAPSSKSTSGGTAALGCLVKDYFPEPVTVSWNSGALTSGVHTFPAVLQSSGLYSLSSVVTVPSSSLGTQTYICNVNHKPSNTKVDKRVEPKSCDKTHTCPPCPAPEAAGGPSVFLFPPKPKDTLMISRTPEVTCVVVDVSHEDPEVKFNWYVDGVEVHNAKTKPREEQYNSTYRVVSVLTVLHQDWLNGKEYKCKVSNKALPAPIEKTISKAKGQPREPQVYTLPPSREEMTKNQVSLTCLVKGFYPSDIAVEWESNGQPENNYKTTPPVLDSDGSFFLYSKLTVDKSRWQQGNVFSCSVMHEALHNHYTQKSLSLSPGK

SEQ ID NO: 147 - protein, 445 aa, Artificial
  heavy chain
QVQLVQSGAEVKKPGASVKVSCKASGYTFTSSYINWVRQAPGQGLEWMGQINAASGMTRYAQKFQGRVTMTRDTSISTAYMELSRLRSDDTAVYYCARGGWFDYWGQGTLVTVSSASTKGPSVFPLAPSSKSTSGGTAALGCLVKDYFPEPVTVSWNSGALTSGVHTFPAVLQSSGLYSLSSVVTVPSSSLGTQTYICNVNHKPSNTKVDKRVEPKSCDKTHTCPPCPAPEAAGGPSVFLFPPKPKDTLMISRTPEVTCVVVDVSHEDPEVKFNWYVDGVEVHNAKTKPREEQYNSTYRVVSVLTVLHQDWLNGKEYKCKVSNKALPAPIEKTISKAKGQPREPQVYTLPPSREEMTKNQVSLTCLVKGFYPSDIAVEWESNGQPENNYKTTPPVLDSDGSFFLYSKLTVDKSRWQQGNVFSCSVMHEALHNHYTQKSLSLSPGK

SEQ ID NO: 148 - protein, 445 aa, Artificial
  heavy chain
QVQLVQSGAEVKKPGASVKVSCKASGYTFTSSYINWVRQAPGQGLEWMGNINAAAGITLYAQKFQGRVTMTRDTSISTAYMELSRLRSDDTAVYYCARGGWFDYWGQGTLVTVSSASTKGPSVFPLAPSSKSTSGGTAALGCLVKDYFPEPVTVSWNSGALTSGVHTFPAVLQSSGLYSLSSVVTVPSSSLGTQTYICNVNHKPSNTKVDKRVEPKSCDKTHTCPPCPAPEAAGGPSVFLFPPKPKDTLMISRTPEVTCVVVDVSHEDPEVKFNWYVDGVEVHNAKTKPREEQYNSTYRVVSVLTVLHQDWLNGKEYKCKVSNKALPAPIEKTISKAKGQPREPQVYTLPPSREEMTKNQVSLTCLVKGFYPSDIAVEWESNGQPENNYKTTPPVLDSDGSFFLYSKLTVDKSRWQQGNVFSCSVMHEALHNHYTQKSLSLSPGK

SEQ ID NO: 149 - protein, 445 aa, Artificial
  heavy chain
QVQLVQSGAEVKKPGASVKVSCKASGYTFTSSYINWVRQAPGQGLEWMGGINPPAGTTSYAQKFQGRVTMTRDTSISTAYMELSRLRSDDTAVYYCARGGWFDYWGQGTLVTVSSASTKGPSVFPLAPSSKSTSGGTAALGCLVKDYFPEPVTVSWNSGALTSGVHTFPAVLQSSGLYSLSSVVTVPSSSLGTQTYICNVNHKPSNTKVDKRVEPKSCDKTHTCPPCPAPEAAGGPSVFLFPPKPKDTLMISRTPEVTCVVVDVSHEDPEVKFNWYVDGVEVHNAKTKPREEQYNSTYRVVSVLTVLHQDWLNGKEYKCKVSNKALPAPIEKTISKAKGQPREPQVYTLPPSREEMTKNQVSLTCLVKGFYPSDIAVEWESNGQPENNYKTTPPVLDSDGSFFLYSKLTVDKSRWQQGNVFSCSVMHEALHNHYTQKSLSLSPGK

SEQ ID NO: 150 - protein, 445 aa, Artificial
  heavy chain
QVQLVQSGAEVKKPGASVKVSCKASGYTFTSSYINWVRQAPGQGLEWMGNINPATGHADYAQKFQGRVTMTRDTSISTAYMELSRLRSDDTAVYYCARGGWFDYWGQGTLVTVSSASTKGPSVFPLAPSSKSTSGGTAALGCLVKDYFPEPVTVSWNSGALTSGVHTFPAVLQSSGLYSLSSVVTVPSSSLGTQTYICNVNHKPSNTKVDKRVEPKSCDKTHTCPPCPAPEAAGGPSVFLFPPKPKDTLMISRTPEVTCVVVDVSHEDPEVKFNWYVDGVEVHNAKTKPREEQYNSTYRVVSVLTVLHQDWLNGKEYKCKVSNKALPAPIEKTISKAKGQPREPQVYTLPPSREEMTKNQVSLTCLVKGFYPSDIAVEWESNGQPENNYKTTPPVLDSDGSFFLYSKLTVDKSRWQQGNVFSCSVMHEALHNHYTQKSLSLSPGK

SEQ ID NO: 151 - protein, 217 aa, Artificial; identical to SEQ ID NO: 141
  light chain

SEQ ID NO: 152 - protein, 217 aa, Artificial; identical to SEQ ID NO: 141
  light chain

SEQ ID NO: 153 - protein, 217 aa, Artificial; identical to SEQ ID NO: 141
  light chain

SEQ ID NO: 154 - protein, 217 aa, Artificial; identical to SEQ ID NO: 141
  light chain

SEQ ID NO: 155 - protein, 217 aa, Artificial; identical to SEQ ID NO: 141
  light chain

SEQ ID NO: 156 - protein, 441 aa, Artificial
  heavy chain
QVQLVQSGAEVKKPGASVKVSCKASGYTFTSSYINWVRQAPGQGLEWMGTINPVSGSTSYAQKFQGRVTMTRDTSISTAYMELSRLRSDDTAVYYCARGGWFDYWGQGTLVTVSSASTKGPSVFPLAPCSRSTSESTAALGCLVKDYFPEPVTVSWNSGALTSGVHTFPAVLQSSGLYSLSSVVTVPSSNFGTQTYTCNVDHKPSNTKVDKTVERKCCVECPPCPAPPVAGPSVFLFPPKPKDTLMISRTPEVTCVVVDVSHEDPEVQFNWYVDGVEVHNAKTKPREEQFNSTFRVVSVLTVVHQDWLNGKEYKCKVSNKGLPAPIEKTISKTKGQPREPQVYTLPPSREEMTKNQVSLTCLVKGFYPSDIAVEWESNGQPENNYKTTPPMLDSDGSFFLYSKLTVDKSRWQQGNVFSCSVMHEALHNHYTQKSLSLSPGK

SEQ ID NO: 157 - protein, 441 aa, Artificial
  heavy chain
QVQLVQSGAEVKKPGASVKVSCKASGYTFTSSYINWVRQAPGQGLEWMGQINAASGMTRYAQKFQGRVTMTRDTSISTAYMELSRLRSDDTAVYYCARGGWFDYWGQGTLVTVSSASTKGPSVFPLAPCSRSTSESTAALGCLVKDYFPEPVTVSWNSGALTSGVHTFPAVLQSSGLYSLSSVVTVPSSNFGTQTYTCNVDHKPSNTKVDKTVERKCCVECPPCPAPPVAGPSVFLFPPKPKDTLMISRTPEVTCVVVDVSHEDPEVQFNWYVDGVEVHNAKTKPREEQFNSTFRVVSVLTVVHQDWLNGKEYKCKVSNKGLPAPIEKTISKTKGQPREPQVYTLPPSREEMTKNQVSLTCLVKGFYPSDIAVEWESNGQPENNYKTTPPMLDSDGSFFLYSKLTVDKSRWQQGNVFSCSVMHEALHNHYTQKSLSLSPGK

SEQ ID NO: 158 - protein, 441 aa, Artificial
  heavy chain
QVQLVQSGAEVKKPGASVKVSCKASGYTFTSSYINWVRQAPGQGLEWMGNINAAAGITLYAQKFQGRVTMTRDTSISTAYMELSRLRSDDTAVYYCARGGWFDYWGQGTLVTVSSASTKGPSVFPLAPCSRSTSESTAALGCLVKDYFPEPVTVSWNSGALTSGVHTFPAVLQSSGLYSLSSVVTVPSSNFGTQTYTCNVDHKPSNTKVDKTVERKCCVECPPCPAPPVAGPSVFLFPPKPKDTLMISRTPEVTCVVVDVSHEDPEVQFNWYVDGVEVHNAKTKPREEQFNSTFRVVSVLTVVHQDWLNGKEYKCKVSNKGLPAPIEKTISKTKGQPREPQVYTLPPSREEMTKNQVSLTCLVKGFYPSDIAVEWESNGQPENNYKTTPPMLDSDGSFFLYSKLTVDKSRWQQGNVFSCSVMHEALHNHYTQKSLSLSPGK

SEQ ID NO: 159 - protein, 441 aa, Artificial
  heavy chain
QVQLVQSGAEVKKPGASVKVSCKASGYTFTSSYINWVRQAPGQGLEWMGGINPPAGTTSYAQKFQGRVTMTRDTSISTAYMELSRLRSDDTAVYYCARGGWFDYWGQGTLVTVSSASTKGPSVFPLAPCSRSTSESTAALGCLVKDYFPEPVTVSWNSGALTSGVHTFPAVLQSSGLYSLSSVVTVPSSNFGTQTYTCNVDHKPSNTKVDKTVERKCCVECPPCPAPPVAGPSVFLFPPKPKDTLMISRTPEVTCVVVDVSHEDPEVQFNWYVDGVEVHNAKTKPREEQFNSTFRVVSVLTVVHQDWLNGKEYKCKVSNKGLPAPIEKTISKTKGQPREPQVYTLPPSREEMTKNQVSLTCLVKGFYPSDIAVEWESNGQPENNYKTTPPMLDSDGSFFLYSKLTVDKSRWQQGNVFSCSVMHEALHNHYTQKSLSLSPGK

SEQ ID NO: 160 - protein, 441 aa, Artificial
  heavy chain
QVQLVQSGAEVKKPGASVKVSCKASGYTFTSSYINWVRQAPGQGLEWMGNINPATGHADYAQKFQGRVTMTRDTSISTAYMELSRLRSDDTAVYYCARGGWFDYWGQGTLVTVSSASTKGPSVFPLAPCSRSTSESTAALGCLVKDYFPEPVTVSWNSGALTSGVHTFPAVLQSSGLYSLSSVVTVPSSNFGTQTYTCNVDHKPSNTKVDKTVERKCCVECPPCPAPPVAGPSVFLFPPKPKDTLMISRTPEVTCVVVDVSHEDPEVQFNWYVDGVEVHNAKTKPREEQFNSTFRVVSVLTVVHQDWLNGKEYKCKVSNKGLPAPIEKTISKTKGQPREPQVYTLPPSREEMTKNQVSLTCLVKGFYPSDIAVEWESNGQPENNYKTTPPMLDSDGSFFLYSKLTVDKSRWQQGNVFSCSVMHEALHNHYTQKSLSLSPGK

SEQ ID NO: 161 - DNA, 651 bp, Artificial
  light chain
cagagcgccctgacccagcccgccagcgtgtccggcagcccaggccagtctatcacaatcagctgcaccggcacctccagcgacgtgggcagctacaactacgtgaactggtatcagcagcaccccggcaaggcccccaagctgatgatctacggcgtgagcaagaggcccagcggcgtgtccaacaggttcagcggcagcaagagcggcaacaccgccagcctgacaatcagtgggctgcaggctgaggacgaggccgactactactgcggcacctttgccggcggatcatactacggcgtgttcggcggagggaccaagctgaccgtgctgggccagcctaaggctgcccccagcgtgaccctgttcccccccagcagcgaggagctgcaggccaacaaggccaccctggtgtgcctgatcagcgacttctacccaggcgccgtgaccgtggcctggaaggccgacagcagccccgtgaaggccggcgtggagaccaccacccccagcaagcagagcaacaacaagtacgccgccagcagctacctgagcctgacccccgagcagtggaagagccacaggtcctacagctgccaggtgacccacgagggcagcaccgtggaaaagaccgtggccccaaccgagtgcagc

SEQ ID NO: 162 - DNA, 651 bp, Artificial; identical to SEQ ID NO: 161
  light chain

SEQ ID NO: 163 - DNA, 651 bp, Artificial
  light chain
cagagcgcactgacccagccagcttcagtgagcggctcaccaggtcagagcattaccatctcgtgtacgggtactagcagcgatgttggttcttataattatgtgaattggtaccagcagcatcccgggaaggcgccgaaacttatgatttatggtgtttctaagcgtccctcaggcgtgagcaaccgttttagcggatccaaaagcggcaacaccgcgagcctgaccattagcggcctgcaagcggaagacgaagcggattattattgcggtacttttgctggtggttcttattatggtgtgtttggcggcggcacgaagttaaccgtcctaggtcagcccaaggctgccccctcggtcactctgttcccgccctcctctgaggagcttcaagccaacaaggccacactggtgtgtctcataagtgacttctacccgggagccgtgacagtggcctggaaggcagatagcagccccgtcaaggcgggagtggagaccaccacaccctccaaacaaagcaacaacaagtacgcggccagcagctatctgagcctgacgcctgagcagtggaagtcccacagaagctacagctgccaggtcacgcatgaagggagcaccgtggagaagacagtggcccctacagaatgttca

SEQ ID NO: 164 - DNA, 651 bp, Artificial; identical to SEQ ID NO: 163
  light chain

SEQ ID NO: 165 - DNA, 651 bp, Artificial; identical to SEQ ID NO: 163
  light chain

SEQ ID NO: 166 - DNA, 1335 bp, Artificial
  heavy chain
caggtgcagctggtgcagagcggagctgaggtgaagaagccaggcgccagcgtcaaggtgtcctgcaaggccagcggctacaccttcaccagcagctacatcaactgggtccgccaggctcctgggcagggactggagtggatgggcaccatcaaccccgtgtccggcagcaccagctacgcccagaagttccagggcagagtcaccatgaccagggacaccagcatcagcaccgcctacatggagctgtccaggctgagaagcgacgacaccgccgtgtactactgcgccaggggcggctggttcgactactggggccagggcaccctggtgaccgtgtcctcagctagcaccaagggccccagcgtgttccccctggcccccagcagcaagagcacctccggcggcacagccgccctgggctgcctggtgaaggactacttccccgagcccgtgaccgtgtcctggaacagcggagccctgaccagcggcgtgcacaccttccccgccgtgctgcagagcagcggcctgtacagcctgtccagcgtggtgacagtgcccagcagcagcctgggcacccagacctacatctgcaacgtgaaccacaagcccagcaacaccaaggtggacaagagagtggagcccaagagctgcgacaagacccacacctgccccccctgcccagcccccgaagctgcaggcggcccttccgtgttcctgttcccccccaagcccaaggacaccctgatgatcagcaggacccccgaggtgacctgcgtggtggtggacgtgagccacgaggacccagaggtgaagttcaactggtacgtggacggcgtggaggtgcacaacgccaagaccaagcccagagaggagcagtacaacagcacctacagggtggtgtccgtgctgaccgtgctgcaccaggactggctgaacggcaaagaatacaagtgcaaggtctccaacaaggccctgcctgcccccatcgaaaagaccatcagcaaggccaagggccagccacgggagccccaggtgtacaccctgcccccttctcgggaggagatgaccaagaaccaggtgtccctgacctgtctggtgaagggcttctaccccagcgacatcgccgtggagtgggagagcaacggccagcccgagaacaactacaagaccacccccccagtgctggacagcgacggcagcttcttcctgtacagcaagctgaccgtggacaagagcaggtggcagcagggcaacgtgttcagctgcagcgtgatgcacgaggccctgcacaaccactacacccagaagagcctgagcctgtcacccggcaag

SEQ ID NO: 167 - DNA, 1335 bp, Artificial
  heavy chain
caggtgcagctggtgcagagcggagctgaggtgaagaagccaggcgccagcgtcaaggtgtcctgcaaggccagcggctacaccttcaccagcagctacatcaactgggtgcgccaggctccagggcagggactggagtggatgggccagatcaacgccgccagcggcatgaccagatacgcccagaagttccagggcagagtcacaatgaccagggacacctctatcagcaccgcctacatggagctgtccaggctgagaagcgacgacaccgccgtgtactactgcgccaggggcggctggttcgactactggggccagggcaccctggtgaccgtgtcctcagctagcaccaagggccccagcgtgttccccctggcccccagcagcaagagcacctccggcggcacagccgccctgggctgcctggtgaaggactacttccccgagcccgtgaccgtgtcctggaacagcggagccctgaccagcggcgtgcacaccttccccgccgtgctgcagagcagcggcctgtacagcctgtccagcgtggtgacagtgcccagcagcagcctgggcacccagacctacatctgcaacgtgaaccacaagcccagcaacaccaaggtggacaagagagtggagcccaagagctgcgacaagacccacacctgccccccctgcccagcccccgaagctgcaggcggcccttccgtgttcctgttcccccccaagcccaaggacaccctgatgatcagcaggacccccgaggtgacctgcgtggtggtggacgtgagccacgaggacccagaggtgaagttcaactggtacgtggacggcgtggaggtgcacaacgccaagaccaagcccagagaggagcagtacaacagcacctacagggtggtgtccgtgctgaccgtgctgcaccaggactggctgaacggcaaagaatacaagtgcaaggtctccaacaaggccctgcctgcccccatcgaaaagaccatcagcaaggccaagggccagccacgggagccccaggtgtacaccctgcccccttctcgggaggagatgaccaagaaccaggtgtccctgacctgtctggtgaagggcttctaccccagcgacatcgccgtggagtgggagagcaacggccagcccgagaacaactacaagaccacccccccagtgctggacagcgacggcagcttcttcctgtacagcaagctgaccgtggacaagagcaggtggcagcagggcaacgtgttcagctgcagcgtgatgcacgaggccctgcacaaccactacacccagaagagcctgagcctgtcacccggcaag

SEQ ID NO: 168 - DNA, 1335 bp, Artificial
  heavy chain
caggtgcaattggttcagagcggcgcggaagtgaaaaaaccgggcgcgagcgtgaaagtgagctgcaaagcctccggatatacctttacttcttcttatattaattgggtccgccaagcccctgggcagggtctcgagtggatgggcaatattaatgctgctgctggtattactctttatgctcagaagtttcagggtcgggtcaccatgacccgtgataccagcattagcaccgcgtatatggaactgagccgcctgcgtagcgatgatacggccgtgtattattgcgcgcgtggtggttggtttgattattggggccaaggcaccctggtgacggttagctcagcctccaccaagggtccatcggtcttccccctggcaccctcctccaagagcacctctgggggcacagcggccctgggctgcctggtcaaggactacttccccgaaccggtgacggtgtcgtggaactcaggcgccctgaccagcggcgtgcacaccttcccggctgtcctacagtcctcaggactctactccctcagcagcgtggtgaccgtgccctccagcagcttgggcacccagacctacatctgcaacgtgaatcacaagcccagcaacaccaaggtggacaagagagttgagcccaaatcttgtgacaaaactcacacatgcccaccgtgcccagcacctgaagcagcggggggaccgtcagtcttcctcttccccccaaaacccaaggacaccctcatgatctcccggacccctgaggtcacatgcgtggtggtggacgtgagccacgaagaccctgaggtcaagttcaactggtacgtggacggcgtggaggtgcataatgccaagacaaagccgcgggaggagcagtacaacagcacgtaccgggtggtcagcgtcctcaccgtcctgcaccaggactggctgaatggcaaggagtacaagtgcaaggtctccaacaaagccctcccagcccccatcgagaaaaccatctccaaagccaaagggcagccccgagaaccacaggtgtacaccctgcccccatcccgggaggagatgaccaagaaccaggtcagcctgacctgcctggtcaaaggcttctatcccagcgacatcgccgtggagtgggagagcaatgggcagccggagaacaactacaagaccacgcctcccgtgctggactccgacggctccttcttcctctacagcaagctcaccgtggacaagagcaggtggcagcaggggaacgtcttctcatgctccgtgatgcatgaggctctgcacaaccactacacgcagaagagcctctccctgtctccgggtaaa

SEQ ID NO: 169 - DNA, 1335 bp, Artificial
  heavy chain
caggtgcaattggttcagagcggcgcggaagtgaaaaaaccgggcgcgagcgtgaaagtgagctgcaaagcctccggatatacctttacttcttcttatattaattgggtccgccaagcccctgggcagggtctcgagtggatgggcggtattaatcctcctgctggtactacttcttatgctcagaagtttcagggtcgggtcaccatgacccgtgataccagcattagcaccgcgtatatggaactgagccgcctgcgtagcgatgatacggccgtgtattattgcgcgcgtggtggttggtttgattattggggccaaggcaccctggtgacggttagctcagcctccaccaagggtccatcggtcttccccctggcaccctcctccaagagcacctctgggggcacagcggccctgggctgcctggtcaaggactacttccccgaaccggtgacggtgtcgtggaactcaggcgccctgaccagcggcgtgcacaccttcccggctgtcctacagtcctcaggactctactccctcagcagcgtggtgaccgtgccctccagcagcttgggcacccagacctacatctgcaacgtgaatcacaagcccagcaacaccaaggtggacaagagagttgagcccaaatcttgtgacaaaactcacacatgcccaccgtgcccagcacctgaagcagcggggggaccgtcagtcttcctcttccccccaaaacccaaggacaccctcatgatctcccggacccctgaggtcacatgcgtggtggtggacgtgagccacgaagaccctgaggtcaagttcaactggtacgtggacggcgtggaggtgcataatgccaagacaaagccgcgggaggagcagtacaacagcacgtaccgggtggtcagcgtcctcaccgtcctgcaccaggactggctgaatggcaaggagtacaagtgcaaggtctccaacaaagccctcccagcccccatcgagaaaaccatctccaaagccaaagggcagccccgagaaccacaggtgtacaccctgcccccatcccgggaggagatgaccaagaaccaggtcagcctgacctgcctggtcaaaggcttctatcccagcgacatcgccgtggagtgggagagcaatgggcagccggagaacaactacaagaccacgcctcccgtgctggactccgacggctccttcttcctctacagcaagctcaccgtggacaagagcaggtggcagcaggggaacgtcttctcatgctccgtgatgcatgaggctctgcacaaccactacacgcagaagagcctctccctgtctccgggtaaa

SEQ ID NO: 170 - DNA, 1335 bp, Artificial
  heavy chain
caggtgcaattggttcagagcggcgcggaagtgaaaaaaccgggcgcgagcgtgaaagtgagctgcaaagcctccggatatacctttacttcttcttatattaattgggtccgccaagcccctgggcagggtctcgagtggatgggcaatattaatcctgctactggtcatgctgattatgctcagaagtttcagggtcgggtgaccatgacccgtgataccagcattagcaccgcgtatatggaactgagccgcctgcgtagcgatgatacggccgtgtattattgcgcgcgtggtggttggtttgattattggggccaaggcaccctggtgacggttagctcagcctccaccaagggtccatcggtcttccccctggcaccctcctccaagagcacctctgggggcacagcggccctgggctgcctggtcaaggactacttccccgaaccggtgacggtgtcgtggaactcaggcgccctgaccagcggcgtgcacaccttcccggctgtcctacagtcctcaggactctactccctcagcagcgtggtgaccgtgccctccagcagcttgggcacccagacctacatctgcaacgtgaatcacaagcccagcaacaccaaggtggacaagagagttgagcccaaatcttgtgacaaaactcacacatgcccaccgtgcccagcacctgaagcagcggggggaccgtcagtcttcctcttccccccaaaacccaaggacaccctcatgatctcccggacccctgaggtcacatgcgtggtggtggacgtgagccacgaagaccctgaggtcaagttcaactggtacgtggacggcgtggaggtgcataatgccaagacaaagccgcgggaggagcagtacaacagcacgtaccgggtggtcagcgtcctcaccgtcctgcaccaggactggctgaatggcaaggagtacaagtgcaaggtctccaacaaagccctcccagcccccatcgagaaaaccatctccaaagccaaagggcagccccgagaaccacaggtgtacaccctgcccccatcccgggaggagatgaccaagaaccaggtcagcctgacctgcctggtcaaaggcttctatcccagcgacatcgccgtggagtgggagagcaatgggcagccggagaacaactacaagaccacgcctcccgtgctggactccgacggctccttcttcctctacagcaagctcaccgtggacaagagcaggtggcagcaggggaacgtcttctcatgctccgtgatgcatgaggctctgcacaaccactacacgcagaagagcctctccctgtctccgggtaaa

SEQ ID NO: 171 - DNA, 651 bp, Artificial; identical to SEQ ID NO: 161
  light chain

SEQ ID NO: 172 - DNA, 651 bp, Artificial; identical to SEQ ID NO: 161
  light chain

SEQ ID NO: 173 - DNA, 651 bp, Artificial; identical to SEQ ID NO: 163
  light chain

SEQ ID NO: 174 - DNA, 651 bp, Artificial; identical to SEQ ID NO: 163
  light chain

SEQ ID NO: 175 - DNA, 651 bp, Artificial; identical to SEQ ID NO: 163
  light chain

SEQ ID NO: 176 - DNA, 1323 bp, Artificial
  heavy chain
caggtgcagctggtgcagagcggagctgaggtgaagaagccaggcgccagcgtcaaggtgtcctgcaaggccagcggctacaccttcaccagcagctacatcaactgggtccgccaggctcctgggcagggactggagtggatgggcaccatcaaccccgtgtccggcagcaccagctacgcccagaagttccagggcagagtcaccatgaccagggacaccagcatcagcaccgcctacatggagctgtccaggctgagaagcgacgacaccgccgtgtactactgcgccaggggcggctggttcgactactggggccagggcaccctggtgaccgtgtcctcagctagcaccaagggccccagcgtgttccccctggccccctgcagcagaagcaccagcgagagcacagccgccctgggctgcctggtgaaggactacttccccgagccagtgaccgtgtcctggaacagcggagccctgaccagcggcgtgcacaccttccccgccgtgctgcagagcagcggcctgtacagcctgtccagcgtggtgaccgtgcccagcagcaacttcggcacccagacctacacctgcaacgtggaccacaagcccagcaacaccaaggtggacaagaccgtggagaggaagtgctgcgtggagtgccccccctgcccagcccccccagtggccggaccctccgtgttcctgttcccccccaagcccaaggacaccctgatgatcagcaggacccccgaggtgacctgcgtggtggtggacgtgagccacgaggacccagaggtgcagttcaactggtacgtggacggcgtggaggtgcacaacgccaagaccaagcccagagaggaacagtttaacagcaccttcagggtggtgtccgtgctgaccgtggtgcaccaggactggctgaacggcaaagagtacaagtgcaaggtctccaacaagggcctgccagcccccatcgagaaaaccatcagcaagaccaagggccagccacgggagccccaggtgtacaccctgccccccagccgggaggaaatgaccaagaaccaggtgtccctgacctgtctggtgaagggcttctaccccagcgacatcgccgtggagtgggagagcaacggccagcccgagaacaactacaagaccaccccccccatgctggacagcgacggcagcttcttcctgtacagcaagctgacagtggacaagagcaggtggcagcagggcaacgtgttcagctgcagcgtgatgcacgaggccctgcacaaccactacacccagaagagcctgagcctgtcccccggcaag

SEQ ID NO: 177 - DNA, 1323 bp, Artificial
  heavy chain
caggtgcagctggtgcagagcggagctgaggtgaagaagccaggcgccagcgtcaaggtgtcctgcaaggccagcggctacaccttcaccagcagctacatcaactgggtgcgccaggctccagggcagggactggagtggatgggccagatcaacgccgccagcggcatgaccagatacgcccagaagttccagggcagagtcacaatgaccagggacacctctatcagcaccgcctacatggagctgtccaggctgagaagcgacgacaccgccgtgtactactgcgccaggggcggctggttcgactactggggccagggcaccctggtgaccgtgtcctcagctagcaccaagggccccagcgtgttccccctggccccctgcagcagaagcaccagcgagagcacagccgccctgggctgcctggtgaaggactacttccccgagccagtgaccgtgtcctggaacagcggagccctgaccagcggcgtgcacaccttccccgccgtgctgcagagcagcggcctgtacagcctgtccagcgtggtgaccgtgcccagcagcaacttcggcacccagacctacacctgcaacgtggaccacaagcccagcaacaccaaggtggacaagaccgtggagaggaagtgctgcgtggagtgccccccctgcccagcccccccagtggccggaccctccgtgttcctgttcccccccaagcccaaggacaccctgatgatcagcaggacccccgaggtgacctgcgtggtggtggacgtgagccacgaggacccagaggtgcagttcaactggtacgtggacggcgtggaggtgcacaacgccaagaccaagcccagagaggaacagtttaacagcaccttcagggtggtgtccgtgctgaccgtggtgcaccaggactggctgaacggcaaagagtacaagtgcaaggtctccaacaagggcctgccagcccccatcgagaaaaccatcagcaagaccaagggccagccacgggagccccaggtgtacaccctgccccccagccgggaggaaatgaccaagaaccaggtgtccctgacctgtctggtgaagggcttctaccccagcgacatcgccgtggagtgggagagcaacggccagcccgagaacaactacaagaccaccccccccatgctggacagcgacggcagcttcttcctgtacagcaagctgacagtggacaagagcaggtggcagcagggcaacgtgttcagctgcagcgtgatgcacgaggccctgcacaaccactacacccagaagagcctgagcctgtcccccggcaag

SEQ ID NO: 178 - DNA, 1323 bp, Artificial
  heavy chain
caggtgcaattggttcagagcggcgcggaagtgaaaaaaccgggcgcgagcgtgaaagtgagctgcaaagcctccggatatacctttacttcttcttatattaattgggtccgccaagcccctgggcagggtctcgagtggatgggcaatattaatgctgctgctggtattactctttatgctcagaagtttcagggtcgggtcaccatgacccgtgataccagcattagcaccgcgtatatggaactgagccgcctgcgtagcgatgatacggccgtgtattattgcgcgcgtggtggttggtttgattattggggccaaggcaccctggtgacggttagctcagcttccaccaagggccccagcgtgttccccctggccccctgcagcagaagcaccagcgagagcacagccgccctgggctgcctggtgaaggactacttccccgagcccgtgaccgtgagctggaacagcggagccctgaccagcggcgtgcacaccttccccgccgtgctgcagagcagcggcctgtacagcctgagcagcgtggtgaccgtgcccagcagcaacttcggcacccagacctacacctgcaacgtggaccacaagcccagcaacaccaaggtggacaagaccgtggagcggaagtgctgcgtggagtgccccccctgccctgcccctcctgtggccggaccctccgtgttcctgttcccccccaagcccaaggacaccctgatgatcagccggacccccgaggtgacctgcgtggtggtggacgtgagccacgaggaccccgaggtgcagttcaactggtacgtggacggcgtggaggtgcacaacgccaagaccaagccccgggaggaacagttcaacagcaccttccgggtggtgtccgtgctgaccgtggtgcaccaggactggctgaacggcaaagaatacaagtgcaaggtgtccaacaagggcctgcctgcccccatcgagaaaaccatcagcaagacaaagggccagcccagggaaccccaggtgtacaccctgccccccagccgggaggaaatgaccaagaaccaggtgtccctgacctgtctggtgaagggcttctaccccagcgacatcgccgtggagtgggagagcaacggccagcccgagaacaactacaagaccaccccccccatgctggacagcgacggcagcttcttcctgtacagcaagctgacagtggacaagagccggtggcagcagggcaacgtgttcagctgcagcgtgatgcacgaggccctgcacaaccactacacccagaagagcctgagcctgtcccccggcaaa

SEQ ID NO: 179 - DNA, 1323 bp, Artificial
  heavy chain
caggtgcaattggttcagagcggcgcggaagtgaaaaaaccgggcgcgagcgtgaaagtgagctgcaaagcctccggatatacctttacttcttcttatattaattgggtccgccaagcccctgggcagggtctcgagtggatgggcggtattaatcctcctgctggtactacttcttatgctcagaagtttcagggtcgggtcaccatgacccgtgataccagcattagcaccgcgtatatggaactgagccgcctgcgtagcgatgatacggccgtgtattattgcgcgcgtggtggttggtttgattattggggccaaggcaccctggtgacggttagctcagcttccaccaagggccccagcgtgttccccctggccccctgcagcagaagcaccagcgagagcacagccgccctgggctgcctggtgaaggactacttccccgagcccgtgaccgtgagctggaacagcggagccctgaccagcggcgtgcacaccttccccgccgtgctgcagagcagcggcctgtacagcctgagcagcgtggtgaccgtgcccagcagcaacttcggcacccagacctacacctgcaacgtggaccacaagcccagcaacaccaaggtggacaagaccgtggagcggaagtgctgcgtggagtgccccccctgccctgcccctcctgtggccggaccctccgtgttcctgttcccccccaagcccaaggacaccctgatgatcagccggacccccgaggtgacctgcgtggtggtggacgtgagccacgaggaccccgaggtgcagttcaactggtacgtggacggcgtggaggtgcacaacgccaagaccaagccccgggaggaacagttcaacagcaccttccgggtggtgtccgtgctgaccgtggtgcaccaggactggctgaacggcaaagaatacaagtgcaaggtgtccaacaagggcctgcctgcccccatcgagaaaaccatcagcaagacaaagggccagcccagggaaccccaggtgtacaccctgccccccagccgggaggaaatgaccaagaaccaggtgtccctgacctgtctggtgaagggcttctaccccagcgacatcgccgtggagtgggagagcaacggccagcccgagaacaactacaagaccaccccccccatgctggacagcgacggcagcttcttcctgtacagcaagctgacagtggacaagagccggtggcagcagggcaacgtgttcagctgcagcgtgatgcacgaggccctgcacaaccactacacccagaagagcctgagcctgtcccccggcaaa

SEQ ID NO: 180 - DNA, 1323 bp, Artificial
  heavy chain
caggtgcaattggttcagagcggcgcggaagtgaaaaaaccgggcgcgagcgtgaaagtgagctgcaaagcctccggatatacctttacttcttcttatattaattgggtccgccaagcccctgggcagggtctcgagtggatgggcaatattaatcctgctactggtcatgctgattatgctcagaagtttcagggtcgggtgaccatgacccgtgataccagcattagcaccgcgtatatggaactgagccgcctgcgtagcgatgatacggccgtgtattattgcgcgcgtggtggttggtttgattattggggccaaggcaccctggtgacggttagctcagcttccaccaagggccccagcgtgttccccctggccccctgcagcagaagcaccagcgagagcacagccgccctgggctgcctggtgaaggactacttccccgagcccgtgaccgtgagctggaacagcggagccctgaccagcggcgtgcacaccttccccgccgtgctgcagagcagcggcctgtacagcctgagcagcgtggtgaccgtgcccagcagcaacttcggcacccagacctacacctgcaacgtggaccacaagcccagcaacaccaaggtggacaagaccgtggagcggaagtgctgcgtggagtgccccccctgccctgcccctcctgtggccggaccctccgtgttcctgttcccccccaagcccaaggacaccctgatgatcagccggacccccgaggtgacctgcgtggtggtggacgtgagccacgaggaccccgaggtgcagttcaactggtacgtggacggcgtggaggtgcacaacgccaagaccaagccccgggaggaacagttcaacagcaccttccgggtggtgtccgtgctgaccgtggtgcaccaggactggctgaacggcaaagaatacaagtgcaaggtgtccaacaagggcctgcctgcccccatcgagaaaaccatcagcaagacaaagggccagcccagggaaccccaggtgtacaccctgccccccagccgggaggaaatgaccaagaaccaggtgtccctgacctgtctggtgaagggcttctaccccagcgacatcgccgtggagtgggagagcaacggccagcccgagaacaactacaagaccaccccccccatgctggacagcgacggcagcttcttcctgtacagcaagctgacagtggacaagagccggtggcagcagggcaacgtgttcagctgcagcgtgatgcacgaggccctgcacaaccactacacccagaagagcctgagcctgtcccccggcaaa

SEQ ID NO: 181 - protein, 512 aa, Homo sapiens [sequence omitted]

SEQ ID NO: 182 - protein, 116 aa, Homo sapiens
SGRGEAETRECIYYNANWELERTNQSGLERCEGEQDKRLHCYASWRNSSGTIELVKKGCWLDDFNCYDRQECVATEENPQVYFCCCEGNFCNERFTHLPEAGGPEVTYEPPPTAPT

SEQ ID NO: 183 - protein, 15 aa, Homo sapiens
IELVKKGSWLDDFNS

SEQ ID NO: 184 - protein, 15 aa, Homo sapiens
VKKGSWLDDFNSYDR

SEQ ID NO: 185 - protein, 15 aa, Homo sapiens
GSWLDDFNSYDRQES

SEQ ID NO: 186 - protein, 9 aa, Homo sapiens
GCWLDDFNC

SEQ ID NO: 187 - protein, 15 aa, Homo sapiens
CEGEQDKRLHCYASW

SEQ ID NO: 188 - protein, 6 aa, Homo sapiens
WLDDFN

SEQ ID NO: 189 - protein, 5 aa, Homo sapiens
EQDKR

SEQ ID NO: 190 - protein, 11 aa, Homo sapiens
KGCWLDDFNCY

SEQ ID NO: 191 - protein, 13 aa, Human
CIYYNANWELERT

SEQ ID NO: 192 - protein, 11 aa, Human
YFCCCEGNFCN

SEQ ID NO: 193 - protein, 216 aa, Artificial Sequence
  Light Chain
DIALTQPASVSGSPGQSITISCTGTSSDVGSYNYVNWYQQHPGKAPKLMIYGVSKRPSGVSNRFSGSKSGNTASLTISGLQAEDEADYYCGTFAGGSYYGVFGGGTKLTVLGQPKSTPTLTVFPPSSEELKENKATLVCLISNFSPSGVTVAWKANGTPITQGVDTSNPTKEGNKFMASSFLHLTSDQWRSHNSFTCQVTHEGDTVEKSLSPAECL

SEQ ID NO: 194 - protein, 445 aa, Artificial
  Heavy Chain
QVQLVQSGAEVKKPGASVKVSCKASGYTFTSSYINWVRQAPGQGLEWMGTINPVSGSTSYAQKFQGRVTMTRDTSISTAYMELSSLRSEDTAVYYCARGGWFDYWGQGTLVTVSSAKTTAPSVYPLAPVCGDTTGSSVTLGCLVKGYFPEPVTLTWNSGSLSSGVHTFPAVLQSDLYTLSSSVTVTSSTWPSQSITCNVAHPASSTKVDKKIEPRGPTIKPCPPCKCPAPNAAGGPSVFIFPPKIKDVLMISLSPIVTCVVVDVSEDDPDVQISWFVNNVEVHTAQTQTHREDYNSTLRVVSALPIQHQDWMSGKEFKCKVNNKDLPAPIERTISKPKGSVRAPQVYVLPPPEEEMTKKQVTLTCMVTDFMPEDIYVEWTNNGKTELNYKNTEPVLDSDGSYFMYSKLRVEKKNWVERNSYSCSVVHEGLHNHHTTKSFSRTPGK